European Patent Application EP 4 606 389 A1, published August 27, 2025. Title: UNIQUE METHOXY-PEGYLATED METHIONINE GRANULOCYTE COLONY STIMULATING FACTOR, METHODS OF USE AND PREPARATION THEREOF. Applicant: Ko-Chung Lin. Application WO. The sequence listing filed with the application follows.

SEQUENCE LISTING (3 sequences)

SEQ ID NO: 1 - protein, 175 aa, synthetic construct
MTPLGPASSLPQSFLLKCLEQVRKIQGDGAALQEKLCATYKLCHPEELVLLGHSLGIPWAPLSSCPSQALQLAGCLSQLHSGLFLYQGLLQALEGISPELGPTLDTLQLDVADFATTIWQQMEELGMAPALQPTQGAMPAFASAFQRRAGGVLVASHLQSFLEVSYRVLRHLAQP

SEQ ID NO: 2 - protein, 174 aa, Homo sapiens
TPLGPASSLPQSFLLKCLEQVRKIQGDGAALQEKLCATYKLCHPEELVLLGHSLGIPWAPLSSCPSQALQLAGCLSQLHSGLFLYQGLLQALEGISPELGPTLDTLQLDVADFATTIWQQMEELGMAPALQPTQGAMPAFASAFQRRAGGVLVASHLQSFLEVSYRVLRHLAQP

SEQ ID NO: 3 - DNA, 534 bp, synthetic construct
  source 1..534: mol_type = other DNA
atgactccacttggtccagcaagcagcctgccgcagagcttcctgctgaaatgcctggagcaagttcgtaaaatccaaggtgacggtgcggcgctgcaggagaagctgtgcgcgacctacaaactgtgccacccggaggaactggtgctgctgggtcacagcctgggcatcccgtgggcgccgctgagcagctgcccgagccaggcgctgcaactggcgggttgcctgagccagctgcacagcggtctgttcctgtatcagggcctgctgcaagcgctggagggtatcagcccggaactgggtccgaccctggacaccctgcaactggacgttgcggattttgcgaccaccatttggcagcaaatggaagaactgggtatggcgccggcgctgcagccgacccaaggtgcgatgccggcgttcgcgagcgcgtttcaacgtcgtgcgggtggcgtgctggttgcgagccacctgcagagctttctggaagtgagctaccgtgtgctgcgtcacctggcgcaaccgtaataataa